European Patent Specification EP 3 191 589 B1, published November 26, 2025. Title: FLAVIVIRUS VIRUS LIKE PARTICLE. Applicant: VLP THERAPEUTICS, LLP. The sequence listing filed with the application follows.

SEQUENCE LISTING (24 sequences)

SEQ ID NO: 1 - DNA, 5498 bp, Dengue virus
  misc_feature: DENV1 prM E (Env F108A)
  CDS (1046)..(3073)
tcgcgcgtttcggtgatgacggtgaaaacctctgacacatgcagctcccggagacggtcacagcttgtctgtaagcggatgccgggagcagacaagcccgtcagggcgcgtcagcgggtgttggcgggtgtcggggctggcttaactatgcggcatcagagcagattgtactgagagtgcaccatatgcggtgtgaaataccgcacagatgcgtaaggagaaaataccgcatcaggcgccattcgccattcaggctgcgcaactgttgggaagggcgatcggtgcgggcctcttcgctattacgccagctggcgaaagggggatgtgctgcaaggcgattaagttgggtaacgccagggttttcccagtcacgacgttgtaaaacgacggccagtgaattgacgcgtttgacattgattattgactagttattaatagtaatcaattacggggtcattagttcatagcccatatatggagttccgcgttacataacttacggtaaatggcccgcctggctgaccgcccaacgacccccgcccattgacgtcaataatgacgtatgttcccatagtaacgccaatagggactttccattgacgtcaatgggtggagtatttacggtaaactgcccacttggcagtacatcaagtgtatcatatgccaagtacgccccctattgacgtcaatgacggtaaatggcccgcctggcattatgcccagtacatgaccttatgggactttcctacttggcagtacatctacgtattagtcatcgctattaccatggtgatgcggttttggcagtacatcaatgggcgtggatagcggtttgactcacggggatttccaagtctccaccccattgacgtcaatgggagtttgttttggcaccaaaatcaacgggactttccaaaatgtcgtaacaactccgccccattgacgcaaatgggcggtaggcgtgtacggtgggaggtctatataagcagagctcgtttagtgaaccgtcagataactgcaggtcgacgatatcgcggccgccaccatgtcggtgaccatgctcctcatgctgctgcccacagccctggcgttccatctgaccacccgagggggagagccgcacatgatagttagcaagcaggaaagaggaaaatcacttttgtttaagacctctgcaggtgtcaacatgtgcacccttattgcaatggatttgggagagttatgtgaggacacaatgacctacaaatgcccccggatcactgagacggaaccagatgacgttgactgttggtgcaatgccacggagacatgggtgacctatggaacatgttctcaaactggtgaacaccgacgagacaaacgttccgtcgcactggcaccacacgtagggcttggtctagaaacaagaaccgaaacgtggatgtcctctgaaggcgcttggaaacaaatacaaaaagtggagacctgggctctgagacacccaggattcacggtgatagccctttttctagcacatgccataggaacatccatcacccagaaagggatcatttttattttgctgatgctggtaactccatccatggccatgcggtgcgtgggaataggcaacagagacttcgtggaaggactgtcaggagctacgtgggtggatgtggtactggagcatggaagttgcgtcactaccatggcaaaagacaaaccaacactggacattgaactcttgaagacggaggtcacaaaccctgccgtcctgcgcaaactgtgcattgaagctaaaatatcaaacaccaccaccgattcgagatgtccaacacaaggagaagccacgctggtggaagaacaggacacgaactttgtgtgtcgacgaacgttcgtggacagaggctggggcaatggttgtgggctagccggaaaaggtagcttaataacgtgtgctaagtttaagtgtgtgacaaaactggaaggaaagatagtccaatatgaaaacttaaaatattcagtgatagtcaccgtacacactggagaccagcaccaagttggaaatgagaccacagaacatggaacaactgcaaccataacacctcaagctcccacgtcggaaatacagctgacagactacggagctctaacattggattgttcacctagaacagggctagactttaatgagatggtgttgttgacaatggaaaaaaaatcatggctcgtccacaaacaatggtttctagacttaccactgccttggacctcgggggcttcaacatcccaagagacttggaatagacaagacttgctggtcacatttaagacagctcatgcaaaaaagcaggaagtagtcgtactaggatcacaagaaggagcaatgcacactgcgttgactggagcgacagaaatccaaacgtctggaacgacaacaatttttgcaggacacctgaaatgcagactaaaaatggataaactgactttaaaagggatgtcatatgtaatgtgcacagggtcattcaagttagagaaggaagtggctgagacccagcatggaactgttctagtgcaggttaaatacgaaggaacagatgcaccatgcaagatccccttctcgtcccaagatgagaagggagtaacccagaatgggagattgataacagccaaccccatagtcactgacaaagaaaaaccagtcaacattgaagcggagccaccttttggtgagagctacattgtggtaggagcaggtgaaaaagctttgaaactaagctggttcaagaagggaagcagtatagggaaaatgtttgaagcaactgcccgtggagcacgaaggatggccatcctgggagacactgcatgggacttcggttctataggaggggtgttcacgtctgtgggaaaactgatacaccagatttttgggactgcgtatggagttttgttcagcggtgtttcttggaccatgaagataggaatagggattctgctgacatggctaggattaaactcaaggagcacgtccctttcaatgacgtgtatcgcagttggcatggtcacgctgtacctaggagtcatggttcaggcgtaataaagatctgctgtgccttctagttgccagccatctgttgtttgcccctcccccgtgccttccttgaccctggaaggtgccactcccactgtcctttcctaataaaatgaggaaattgcatcgcattgtctgagtaggtgtcattctattctggggggtggggtggggcaggacagcaagggggaggattgggaagacaatagcaggcatgctggggatgcggtgggctctatggctcgagcatggtcatagctgtttcctgtgtgaaattgttatccgctcacaattccacacaacatacgagccggaagcataaagtgtaaagcctggggtgcctaatgagtgagctaactcacattaattgcgttgcgctcactgcccgctttccagtcgggaaacctgtcgtgccagctgcattaatgaatcggccaacgcgcggggagaggcggtttgcgtattgggcgctcttccgcttcctcgctcactgactcgctgcgctcggtcgttcggctgcggcgagcggtatcagctcactcaaaggcggtaatacggttatccacagaatcaggggataacgcaggaaagaacatgtgagcaaaaggccagcaaaaggccaggaaccgtaaaaaggccgcgttgctggcgtttttccataggctccgcccccctgacgagcatcacaaaaatcgacgctcaagtcagaggtggcgaaacccgacaggactataaagataccaggcgtttccccctggaagctccctcgtgcgctctcctgttccgaccctgccgcttaccggatacctgtccgcctttctcccttcgggaagcgtggcgctttctcatagctcacgctgtaggtatctcagttcggtgtaggtcgttcgctccaagctgggctgtgtgcacgaaccccccgttcagcccgaccgctgcgccttatccggtaactatcgtcttgagtccaacccggtaagacacgacttatcgccactggcagcagccactggtaacaggattagcagagcgaggtatgtaggcggtgctacagagttcttgaagtggtggcctaactacggctacactagaagaacagtatttggtatctgcgctctgctgaagccagttaccttcggaaaaagagttggtagctcttgatccggcaaacaaaccaccgctggtagcggtggtttttttgtttgcaagcagcagattacgcgcagaaaaaaaggatctcaagaagatcctttgatcttttctacggggtctgacgctcagtggaacgaaaactcacgttaagggattttggtcatgagattatcaaaaaggatcttcacctagatccttttaaattaaaaatgaagttttaaatcaatctaaagtatatatgagtaaacttggtctgacagttagaaaaactcatcgagcatcaaatgaaactgcaatttattcatatcaggattatcaataccatatttttgaaaaagccgtttctgtaatgaaggagaaaactcaccgaggcagttccataggatggcaagatcctggtatcggtctgcgattccgactcgtccaacatcaatacaacctattaatttcccctcgtcaaaaataaggttatcaagtgagaaatcaccatgagtgacgactgaatccggtgagaatggcaaaagtttatgcatttctttccagacttgttcaacaggccagccattacgctcgtcatcaaaatcactcgcatcaaccaaaccgttattcattcgtgattgcgcctgagcgagacgaaatacgcgatcgctgttaaaaggacaattacaaacaggaatcgaatgcaaccggcgcaggaacactgccagcgcatcaacaatattttcacctgaatcaggatattcttctaatacctggaatgctgttttcccagggatcgcagtggtgagtaaccatgcatcatcaggagtacggataaaatgcttgatggtcggaagaggcataaattccgtcagccagtttagtctgaccatctcatctgtaacatcattggcaacgctacctttgccatgtttcagaaacaactctggcgcatcgggcttcccatacaatcgatagattgtcgcacctgattgcccgacattatcgcgagcccatttatacccatataaatcagcatccatgttggaatttaatcgcggcctagagcaagacgtttcccgttgaatatggctcatactcttcctttttcaatattattgaagcatttatcagggttattgtctcatgagcggatacatatttgaatgtatttagaaaaataaacaaataggggttccgcgcacatttccccgaaaagtgccacctgacgtctaagaaaccattattatcatgacattaacctataaaaataggcgtatcacgaggccctttcgtc

SEQ ID NO: 2 - protein, 676 aa, Dengue virus
MSVTMLLMLLPTALAFHLTTRGGEPHMIVSKQERGKSLLFKTSAGVNMCTLIAMDLGELCEDTMTYKCPRITETEPDDVDCWCNATETWVTYGTCSQTGEHRRDKRSVALAPHVGLGLETRTETWMSSEGAWKQIQKVETWALRHPGFTVIALFLAHAIGTSITQKGIIFILLMLVTPSMAMRCVGIGNRDFVEGLSGATWVDVVLEHGSCVTTMAKDKPTLDIELLKTEVTNPAVLRKLCIEAKISNTTTDSRCPTQGEATLVEEQDTNFVCRRTFVDRGWGNGCGLAGKGSLITCAKFKCVTKLEGKIVQYENLKYSVIVTVHTGDQHQVGNETTEHGTTATITPQAPTSEIQLTDYGALTLDCSPRTGLDFNEMVLLTMEKKSWLVHKQWFLDLPLPWTSGASTSQETWNRQDLLVTFKTAHAKKQEVVVLGSQEGAMHTALTGATEIQTSGTTTIFAGHLKCRLKMDKLTLKGMSYVMCTGSFKLEKEVAETQHGTVLVQVKYEGTDAPCKIPFSSQDEKGVTQNGRLITANPIVTDKEKPVNIEAEPPFGESYIVVGAGEKALKLSWFKKGSSIGKMFEATARGARRMAILGDTAWDFGSIGGVFTSVGKLIHQIFGTAYGVLFSGVSWTMKIGIGILLTWLGLNSRSTSLSMTCIAVGMVTLYLGVMVQA

SEQ ID NO: 3 - DNA, 5498 bp, Dengue virus
  misc_feature: DENV1 prM E (Env K203N)
  CDS (1046)..(3073)
tcgcgcgtttcggtgatgacggtgaaaacctctgacacatgcagctcccggagacggtcacagcttgtctgtaagcggatgccgggagcagacaagcccgtcagggcgcgtcagcgggtgttggcgggtgtcggggctggcttaactatgcggcatcagagcagattgtactgagagtgcaccatatgcggtgtgaaataccgcacagatgcgtaaggagaaaataccgcatcaggcgccattcgccattcaggctgcgcaactgttgggaagggcgatcggtgcgggcctcttcgctattacgccagctggcgaaagggggatgtgctgcaaggcgattaagttgggtaacgccagggttttcccagtcacgacgttgtaaaacgacggccagtgaattgacgcgtttgacattgattattgactagttattaatagtaatcaattacggggtcattagttcatagcccatatatggagttccgcgttacataacttacggtaaatggcccgcctggctgaccgcccaacgacccccgcccattgacgtcaataatgacgtatgttcccatagtaacgccaatagggactttccattgacgtcaatgggtggagtatttacggtaaactgcccacttggcagtacatcaagtgtatcatatgccaagtacgccccctattgacgtcaatgacggtaaatggcccgcctggcattatgcccagtacatgaccttatgggactttcctacttggcagtacatctacgtattagtcatcgctattaccatggtgatgcggttttggcagtacatcaatgggcgtggatagcggtttgactcacggggatttccaagtctccaccccattgacgtcaatgggagtttgttttggcaccaaaatcaacgggactttccaaaatgtcgtaacaactccgccccattgacgcaaatgggcggtaggcgtgtacggtgggaggtctatataagcagagctcgtttagtgaaccgtcagataactgcaggtcgacgatatcgcggccgccaccatgtcggtgaccatgctcctcatgctgctgcccacagccctggcgttccatctgaccacccgagggggagagccgcacatgatagttagcaagcaggaaagaggaaaatcacttttgtttaagacctctgcaggtgtcaacatgtgcacccttattgcaatggatttgggagagttatgtgaggacacaatgacctacaaatgcccccggatcactgagacggaaccagatgacgttgactgttggtgcaatgccacggagacatgggtgacctatggaacatgttctcaaactggtgaacaccgacgagacaaacgttccgtcgcactggcaccacacgtagggcttggtctagaaacaagaaccgaaacgtggatgtcctctgaaggcgcttggaaacaaatacaaaaagtggagacctgggctctgagacacccaggattcacggtgatagccctttttctagcacatgccataggaacatccatcacccagaaagggatcatttttattttgctgatgctggtaactccatccatggccatgcggtgcgtgggaataggcaacagagacttcgtggaaggactgtcaggagctacgtgggtggatgtggtactggagcatggaagttgcgtcactaccatggcaaaagacaaaccaacactggacattgaactcttgaagacggaggtcacaaaccctgccgtcctgcgcaaactgtgcattgaagctaaaatatcaaacaccaccaccgattcgagatgtccaacacaaggagaagccacgctggtggaagaacaggacacgaactttgtgtgtcgacgaacgttcgtggacagaggctggggcaatggttgtgggctattcggaaaaggtagcttaataacgtgtgctaagtttaagtgtgtgacaaaactggaaggaaagatagtccaatatgaaaacttaaaatattcagtgatagtcaccgtacacactggagaccagcaccaagttggaaatgagaccacagaacatggaacaactgcaaccataacacctcaagctcccacgtcggaaatacagctgacagactacggagctctaacattggattgttcacctagaacagggctagactttaatgagatggtgttgttgacaatggaaaataaatcatggctcgtccacaaacaatggtttctagacttaccactgccttggacctcgggggcttcaacatcccaagagacttggaatagacaagacttgctggtcacatttaagacagctcatgcaaaaaagcaggaagtagtcgtactaggatcacaagaaggagcaatgcacactgcgttgactggagcgacagaaatccaaacgtctggaacgacaacaatttttgcaggacacctgaaatgcagactaaaaatggataaactgactttaaaagggatgtcatatgtaatgtgcacagggtcattcaagttagagaaggaagtggctgagacccagcatggaactgttctagtgcaggttaaatacgaaggaacagatgcaccatgcaagatccccttctcgtcccaagatgagaagggagtaacccagaatgggagattgataacagccaaccccatagtcactgacaaagaaaaaccagtcaacattgaagcggagccaccttttggtgagagctacattgtggtaggagcaggtgaaaaagctttgaaactaagctggttcaagaagggaagcagtatagggaaaatgtttgaagcaactgcccgtggagcacgaaggatggccatcctgggagacactgcatgggacttcggttctataggaggggtgttcacgtctgtgggaaaactgatacaccagatttttgggactgcgtatggagttttgttcagcggtgtttcttggaccatgaagataggaatagggattctgctgacatggctaggattaaactcaaggagcacgtccctttcaatgacgtgtatcgcagttggcatggtcacgctgtacctaggagtcatggttcaggcgtaataaagatctgctgtgccttctagttgccagccatctgttgtttgcccctcccccgtgccttccttgaccctggaaggtgccactcccactgtcctttcctaataaaatgaggaaattgcatcgcattgtctgagtaggtgtcattctattctggggggtggggtggggcaggacagcaagggggaggattgggaagacaatagcaggcatgctggggatgcggtgggctctatggctcgagcatggtcatagctgtttcctgtgtgaaattgttatccgctcacaattccacacaacatacgagccggaagcataaagtgtaaagcctggggtgcctaatgagtgagctaactcacattaattgcgttgcgctcactgcccgctttccagtcgggaaacctgtcgtgccagctgcattaatgaatcggccaacgcgcggggagaggcggtttgcgtattgggcgctcttccgcttcctcgctcactgactcgctgcgctcggtcgttcggctgcggcgagcggtatcagctcactcaaaggcggtaatacggttatccacagaatcaggggataacgcaggaaagaacatgtgagcaaaaggccagcaaaaggccaggaaccgtaaaaaggccgcgttgctggcgtttttccataggctccgcccccctgacgagcatcacaaaaatcgacgctcaagtcagaggtggcgaaacccgacaggactataaagataccaggcgtttccccctggaagctccctcgtgcgctctcctgttccgaccctgccgcttaccggatacctgtccgcctttctcccttcgggaagcgtggcgctttctcatagctcacgctgtaggtatctcagttcggtgtaggtcgttcgctccaagctgggctgtgtgcacgaaccccccgttcagcccgaccgctgcgccttatccggtaactatcgtcttgagtccaacccggtaagacacgacttatcgccactggcagcagccactggtaacaggattagcagagcgaggtatgtaggcggtgctacagagttcttgaagtggtggcctaactacggctacactagaagaacagtatttggtatctgcgctctgctgaagccagttaccttcggaaaaagagttggtagctcttgatccggcaaacaaaccaccgctggtagcggtggtttttttgtttgcaagcagcagattacgcgcagaaaaaaaggatctcaagaagatcctttgatcttttctacggggtctgacgctcagtggaacgaaaactcacgttaagggattttggtcatgagattatcaaaaaggatcttcacctagatccttttaaattaaaaatgaagttttaaatcaatctaaagtatatatgagtaaacttggtctgacagttagaaaaactcatcgagcatcaaatgaaactgcaatttattcatatcaggattatcaataccatatttttgaaaaagccgtttctgtaatgaaggagaaaactcaccgaggcagttccataggatggcaagatcctggtatcggtctgcgattccgactcgtccaacatcaatacaacctattaatttcccctcgtcaaaaataaggttatcaagtgagaaatcaccatgagtgacgactgaatccggtgagaatggcaaaagtttatgcatttctttccagacttgttcaacaggccagccattacgctcgtcatcaaaatcactcgcatcaaccaaaccgttattcattcgtgattgcgcctgagcgagacgaaatacgcgatcgctgttaaaaggacaattacaaacaggaatcgaatgcaaccggcgcaggaacactgccagcgcatcaacaatattttcacctgaatcaggatattcttctaatacctggaatgctgttttcccagggatcgcagtggtgagtaaccatgcatcatcaggagtacggataaaatgcttgatggtcggaagaggcataaattccgtcagccagtttagtctgaccatctcatctgtaacatcattggcaacgctacctttgccatgtttcagaaacaactctggcgcatcgggcttcccatacaatcgatagattgtcgcacctgattgcccgacattatcgcgagcccatttatacccatataaatcagcatccatgttggaatttaatcgcggcctagagcaagacgtttcccgttgaatatggctcatactcttcctttttcaatattattgaagcatttatcagggttattgtctcatgagcggatacatatttgaatgtatttagaaaaataaacaaataggggttccgcgcacatttccccgaaaagtgccacctgacgtctaagaaaccattattatcatgacattaacctataaaaataggcgtatcacgaggccctttcgtc

SEQ ID NO: 4 - protein, 676 aa, Dengue virus
MSVTMLLMLLPTALAFHLTTRGGEPHMIVSKQERGKSLLFKTSAGVNMCTLIAMDLGELCEDTMTYKCPRITETEPDDVDCWCNATETWVTYGTCSQTGEHRRDKRSVALAPHVGLGLETRTETWMSSEGAWKQIQKVETWALRHPGFTVIALFLAHAIGTSITQKGIIFILLMLVTPSMAMRCVGIGNRDFVEGLSGATWVDVVLEHGSCVTTMAKDKPTLDIELLKTEVTNPAVLRKLCIEAKISNTTTDSRCPTQGEATLVEEQDTNFVCRRTFVDRGWGNGCGLFGKGSLITCAKFKCVTKLEGKIVQYENLKYSVIVTVHTGDQHQVGNETTEHGTTATITPQAPTSEIQLTDYGALTLDCSPRTGLDFNEMVLLTMENKSWLVHKQWFLDLPLPWTSGASTSQETWNRQDLLVTFKTAHAKKQEVVVLGSQEGAMHTALTGATEIQTSGTTTIFAGHLKCRLKMDKLTLKGMSYVMCTGSFKLEKEVAETQHGTVLVQVKYEGTDAPCKIPFSSQDEKGVTQNGRLITANPIVTDKEKPVNIEAEPPFGESYIVVGAGEKALKLSWFKKGSSIGKMFEATARGARRMAILGDTAWDFGSIGGVFTSVGKLIHQIFGTAYGVLFSGVSWTMKIGIGILLTWLGLNSRSTSLSMTCIAVGMVTLYLGVMVQA

SEQ ID NO: 5 - DNA, 3770 bp, Dengue virus
  misc_feature: DENV1 capsid K85A_K86A mutant
  CDS (1046)..(1345)
tcgcgcgtttcggtgatgacggtgaaaacctctgacacatgcagctcccggagacggtcacagcttgtctgtaagcggatgccgggagcagacaagcccgtcagggcgcgtcagcgggtgttggcgggtgtcggggctggcttaactatgcggcatcagagcagattgtactgagagtgcaccatatgcggtgtgaaataccgcacagatgcgtaaggagaaaataccgcatcaggcgccattcgccattcaggctgcgcaactgttgggaagggcgatcggtgcgggcctcttcgctattacgccagctggcgaaagggggatgtgctgcaaggcgattaagttgggtaacgccagggttttcccagtcacgacgttgtaaaacgacggccagtgaattgacgcgtttgacattgattattgactagttattaatagtaatcaattacggggtcattagttcatagcccatatatggagttccgcgttacataacttacggtaaatggcccgcctggctgaccgcccaacgacccccgcccattgacgtcaataatgacgtatgttcccatagtaacgccaatagggactttccattgacgtcaatgggtggagtatttacggtaaactgcccacttggcagtacatcaagtgtatcatatgccaagtacgccccctattgacgtcaatgacggtaaatggcccgcctggcattatgcccagtacatgaccttatgggactttcctacttggcagtacatctacgtattagtcatcgctattaccatggtgatgcggttttggcagtacatcaatgggcgtggatagcggtttgactcacggggatttccaagtctccaccccattgacgtcaatgggagtttgttttggcaccaaaatcaacgggactttccaaaatgtcgtaacaactccgccccattgacgcaaatgggcggtaggcgtgtacggtgggaggtctatataagcagagctcgtttagtgaaccgtcagataactgcaggtcgacgatatcgcggccgccaccatgaacaaccaacggaaaaagacgggtcgaccgtctttcaatatgctgaaacgcgcgagaaaccgcgtgtcaactgtttcacagttggcgaagagattctcaaaaggattgctttcaggccaaggacccatgaaattggtgatggcttttatagcattcctaagatttctagccatacctccaacagcaggaattttggctagatggggctcattcaagaagaatggagcgatcaaagtgttacggggtttcgcggcagaaatctcaaacatgttgaacataatgaacaggaggaaaagataataaagatctgctgtgccttctagttgccagccatctgttgtttgcccctcccccgtgccttccttgaccctggaaggtgccactcccactgtcctttcctaataaaatgaggaaattgcatcgcattgtctgagtaggtgtcattctattctggggggtggggtggggcaggacagcaagggggaggattgggaagacaatagcaggcatgctggggatgcggtgggctctatggctcgagcatggtcatagctgtttcctgtgtgaaattgttatccgctcacaattccacacaacatacgagccggaagcataaagtgtaaagcctggggtgcctaatgagtgagctaactcacattaattgcgttgcgctcactgcccgctttccagtcgggaaacctgtcgtgccagctgcattaatgaatcggccaacgcgcggggagaggcggtttgcgtattgggcgctcttccgcttcctcgctcactgactcgctgcgctcggtcgttcggctgcggcgagcggtatcagctcactcaaaggcggtaatacggttatccacagaatcaggggataacgcaggaaagaacatgtgagcaaaaggccagcaaaaggccaggaaccgtaaaaaggccgcgttgctggcgtttttccataggctccgcccccctgacgagcatcacaaaaatcgacgctcaagtcagaggtggcgaaacccgacaggactataaagataccaggcgtttccccctggaagctccctcgtgcgctctcctgttccgaccctgccgcttaccggatacctgtccgcctttctcccttcgggaagcgtggcgctttctcatagctcacgctgtaggtatctcagttcggtgtaggtcgttcgctccaagctgggctgtgtgcacgaaccccccgttcagcccgaccgctgcgccttatccggtaactatcgtcttgagtccaacccggtaagacacgacttatcgccactggcagcagccactggtaacaggattagcagagcgaggtatgtaggcggtgctacagagttcttgaagtggtggcctaactacggctacactagaagaacagtatttggtatctgcgctctgctgaagccagttaccttcggaaaaagagttggtagctcttgatccggcaaacaaaccaccgctggtagcggtggtttttttgtttgcaagcagcagattacgcgcagaaaaaaaggatctcaagaagatcctttgatcttttctacggggtctgacgctcagtggaacgaaaactcacgttaagggattttggtcatgagattatcaaaaaggatcttcacctagatccttttaaattaaaaatgaagttttaaatcaatctaaagtatatatgagtaaacttggtctgacagttagaaaaactcatcgagcatcaaatgaaactgcaatttattcatatcaggattatcaataccatatttttgaaaaagccgtttctgtaatgaaggagaaaactcaccgaggcagttccataggatggcaagatcctggtatcggtctgcgattccgactcgtccaacatcaatacaacctattaatttcccctcgtcaaaaataaggttatcaagtgagaaatcaccatgagtgacgactgaatccggtgagaatggcaaaagtttatgcatttctttccagacttgttcaacaggccagccattacgctcgtcatcaaaatcactcgcatcaaccaaaccgttattcattcgtgattgcgcctgagcgagacgaaatacgcgatcgctgttaaaaggacaattacaaacaggaatcgaatgcaaccggcgcaggaacactgccagcgcatcaacaatattttcacctgaatcaggatattcttctaatacctggaatgctgttttcccagggatcgcagtggtgagtaaccatgcatcatcaggagtacggataaaatgcttgatggtcggaagaggcataaattccgtcagccagtttagtctgaccatctcatctgtaacatcattggcaacgctacctttgccatgtttcagaaacaactctggcgcatcgggcttcccatacaatcgatagattgtcgcacctgattgcccgacattatcgcgagcccatttatacccatataaatcagcatccatgttggaatttaatcgcggcctagagcaagacgtttcccgttgaatatggctcatactcttcctttttcaatattattgaagcatttatcagggttattgtctcatgagcggatacatatttgaatgtatttagaaaaataaacaaataggggttccgcgcacatttccccgaaaagtgccacctgacgtctaagaaaccattattatcatgacattaacctataaaaataggcgtatcacgaggccctttcgtc

SEQ ID NO: 6 - protein, 100 aa, Dengue virus
MNNQRKKTGRPSFNMLKRARNRVSTVSQLAKRFSKGLLSGQGPMKLVMAFIAFLRFLAIPPTAGILARWGSFKKNGAIKVLRGFAAEISNMLNIMNRRKR

SEQ ID NO: 7 - DNA, 6679 bp, Dengue virus
  misc_feature: Chimera DENV2 prM E_chimeric DENV1 E
  CDS (906)..(2933)
  misc_feature (906)..(2336): DENV2 prM E region
  misc_feature (2337)..(2933): DENV1 E region
gaattcccattgcatacgttgtatccatatcataatatgtacatttatattggctcatgtccaacattaccgccatgttgacattgattattgactagttattaatagtaatcaattacggggtcattagttcatagcccatatatggagttccgcgttacataacttacggtaaatggcccgcctggctgaccgcccaacgacccccgcccattgacgtcaataatgacgtatgttcccatagtaacgccaatagggactttccattgacgtcaatgggtggagtatttacggtaaactgcccacttggcagtacatcaagtgtatcatatgccaagtacgccccctattgacgtcaatgacggtaaatggcccgcctggcattatgcccagtacatgaccttatgggactttcctacttggcagtacatctacgtattagtcatcgctattaccatggtgatgcggttttggcagtacatcaatgggcgtggatagcggtttgactcacggggatttccaagtctccaccccattgacgtcaatgggagtttgttttggcaccaaaatcaacgggactttccaaaatgtcgtaacaactccgccccattgacgcaaatgggcggtaggcgtgtacggtgggaggtctatataagcagagctcgtttagtgaaccgtcagatcgcctggagacgccatccacgctgttttgacctccatagaagacaccgggaccgatccagcctccgttaacggtggagggcagtgtagtctgagcagtactcgttgctgccgcgcgcgccaccagacataatagctgacagactaacagactgttcctttccatgggtcttttctgcagtcaccgtcgtcgacacgtgtgatcagatatcgcggccgccaccatgactgcaggcatgatcatcatgctgattccaacagtgatggcgtttcatctgaccacacgcaacggagaaccacacatgatcgtcagtagacaagaaaaagggaaaagccttctgtttaagacaaaggacggcacgaacatgtgtaccctcatggccatggaccttggtgagttgtgtgaagacacaatcacgtataaatgtccctttctcaagcagaacgaaccagaagacatagattgttggtgcaactccacgtccacatgggtaacttatgggacatgtaccaccacaggagagcacagaagagaaaaaagatcagtggcgcttgttccacacgtgggaatgggattggagacacgaactgaaacatggatgtcatcagaaggggcctggaaacatgcccagagaattgaaacttggattctgagacatccaggctttaccataatggccgcaatcctggcatacaccataggaacgacgcatttccaaagagtcctgatattcatcctactgacagccatcgctccttcaatgacaatgcgctgcataggaatatcaaatagggactttgtggaaggagtgtcaggagggagttgggttgacatagttttagaacatggaagttgtgtgacgacgatggcaaaaaataaaccaacactggactttgaactgataaaaacagaagccaaacaacccgccaccttaaggaagtactgtatagaggctaaactgaccaacacgacaacagactcgcgctgcccaacacaaggggaacccaccctgaatgaagagcaggacaaaaggtttgtctgcaaacattccatggtagacagaggatggggaaatggatgtggattatttggaaaaggaggcatcgtgacctgtgccatgttcacatgcaaaaagaacatggagggaaaaattgtgcagccagaaaacctggaatacactgtcgttataacacctcattcaggggaagaacatgcagtcggaaatgacacaggaaaacatggtaaagaagtcaagataacaccacagagctccatcacagaggcggaactgacaggctatggcactgttacgatggagtgctctccaagaacgggcctcgacttcaatgagatggtgttgctgcaaatgaaagacaaagcttggctggtgcacagacaatggttcctagacctaccgttgccatggctgcccggagcagacacacaaggatcaaattggatacagaaagagacactggtcaccttcaaaaatccccatgcgaaaaaacaggatgttgttgtcttaggctcccaagagggggccatgcatacagcactcacaggggctacggaaatccagatgtcatcaggaaacctgctgttcacaggacatcttaagtgcaggctgagaatggacaaattacaacttaaagggatgtcatatgtaatgtgcacagggtcattcaagttagagaaggaagtggctgagacccagcatggaactgttctagtgcaggttaaatacgaaggaacagatgcaccatgcaagatccccttctcgtcccaagatgagaagggagtaacccagaatgggagattgataacagccaaccccatagtcactgacaaagaaaaaccagtcaacattgaagcggagccaccttttggtgagagctacattgtggtaggagcaggtgaaaaagctttgaaactaagctggttcaagaagggaagcagtatagggaaaatgtttgaagcaactgcccgtggagcacgaaggatggccatcctgggagacactgcatgggacttcggttctataggaggggtgttcacgtctgtgggaaaactgatacaccagatttttgggactgcgtatggagttttgttcagcggtgtttcttggaccatgaagataggaatagggattctgctgacatggctaggattaaactcaaggagcacgtccctttcaatgacgtgtatcgcagttggcatggtcacgctgtacctaggagtcatggttcaggcgtaataaagatctgctgtgccttctagttgccagccatctgttgtttgcccctcccccgtgccttccttgaccctggaaggtgccactcccactgtcctttcctaataaaatgaggaaattgcatcgcattgtctgagtaggtgtcattctattctggggggtggggtggggcaggacagcaagggggaggattgggaagacaatagcaggcatgctggggatgcggtgggctctatgggtacccaggtgctgaagaattgacccggttcctcctgggccagaaagaagcaggcacatccccttctctgtgacacaccctgtccacgcccctggttcttagttccagccccactcataggacactcatagctcaggagggctccgccttcaatcccacccgctaaagtacttggagcggtctctccctccctcatcagcccaccaaaccaaacctagcctccaagagtgggaagaaattaaagcaagataggctattaagtgcagagggagagaaaatgcctccaacatgtgaggaagtaatgagagaaatcatagaattttaaggccatgatttaaggccatcatggcctaagcttgaaaggagataggatcaaagcttggcgtaatcatggtcatagctgtttcctgtgtgaaattgttatccgctcacaattccacacaacatacgagccggaagcataaagtgtaaagcctggggtgcctaatgagtgagctaactcacattaattgcgttgcgctcactgcccgctttccagtcgggaaacctgtcgtgccagctgcattaatgaatcggccaacgcgcggggagaggcggtttgcgtattgggcgctcttccgcttcctcgctcactgactcgctgcgctcggtcgttcggctgcggcgagcggtatcagctcactcaaaggcggtaatacggttatccacagaatcaggggataacgcaggaaagaacatgtgagcaaaaggccagcaaaaggccaggaaccgtaaaaaggccgcgttgctggcgtttttccataggctccgcccccctgacgagcatcacaaaaatcgacgctcaagtcagaggtggcgaaacccgacaggactataaagataccaggcgtttccccctggaagctccctcgtgcgctctcctgttccgaccctgccgcttaccggatacctgtccgcctttctcccttcgggaagcgtggcgctttctcatagctcacgctgtaggtatctcagttcggtgtaggtcgttcgctccaagctgggctgtgtgcacgaaccccccgttcagcccgaccgctgcgccttatccggtaactatcgtcttgagtccaacccggtaagacacgacttatcgccactggcagcagccactggtaacaggattagcagagcgaggtatgtaggcggtgctacagagttcttgaagtggtggcctaactacggctacactagaagaacagtatttggtatctgcgctctgctgaagccagttaccttcggaaaaagagttggtagctcttgatccggcaaacaaaccaccgctggtagcggtggtttttttgtttgcaagcagcagattacgcgcagaaaaaaaggatctcaagaagatcctttgatcttttctacggggtctgacgctcagtggaacgaaaactcacgttaagggattttggtcatgagattatcaaaaaggatcttcacctagatccttttaaattaaaaatgaagttttaaatcaatctaaagtatatatgagtaaacttggtctgacagttaccaatgcttaatcagtgaggcacctatctcagcgatctgtctatttcgttcatccatagttgcctgactccccgtcgtgtagataactacgatacgggagggcttaccatctggccccagtgctgcaatgataccgcgagaaccacgctcaccggctccagatttatcagcaataaaccagccagccggaagggccgagcgcagaagtggtcctgcaactttatccgcctccatccagtctattaattgttgccgggaagctagagtaagtagttcgccagttaatagtttgcgcaacgttgttgccattgctacaggcatcgtggtgtcacgctcgtcgtttggtatggcttcattcagctccggttcccaacgatcaaggcgagttacatgatcccccatgttgtgcaaaaaagcggttagctccttcggtcctccgatcgttgtcagaagtaagttggccgcagtgttatcactcatggttatggcagcactgcataattctcttactgtcatgccatccgtaagatgcttttctgtgactggtgagtactcaaccaagtcattctgagaatagtgtatgcggcgaccgagttgctcttgcccggcgtcaatacgggataataccgcgccacatagcagaactttaaaagtgctcatcattggaaaacgttcttcggggcgaaaactctcaaggatcttaccgctgttgagatccagttcgatgtaacccactcgtgcacccaactgatcttcagcatcttttactttcaccagcgtttctgggtgagcaaaaacaggaaggcaaaatgccgcaaaaaagggaataagggcgacacggaaatgttgaatactcatactcttcctttttcaatattattgaagcatttatcagggttattgtctcatgagcggatacatatttgaatgtatttagaaaaataaacaaataggggttccgcgcacatttccccgaaaagtgccacctgacgtctaagaaaccattattatcatgacattaacctataaaaataggcgtatcacgaggccctttcgggtcgcgcgtttcggtgatgacggtgaaaacctctgacacatgcagctcccgttgacggtcacagcttgtctgtaagcggatgccgggagcagacaagcccgtcagggcgcgtcagcgggtgttggcgggtgtcggggctggcttaactatgcggcatcagagcagattgtactgagagtgcaccataaaattgtaaacgttaatattttgttaaaattcgcgttaaatttttgttaaatcagctcattttttaaccaataggccgaaatcggcaaaatcccttataaatcaaaagaatagcccgagatagggttgagtgttgttccagtttggaacaagagtccactattaaagaacgtggactccaacgtcaaagggcgaaaaaccgtctatcagggcgatggcccactacgtgaaccatcacccaaatcaagttttttggggtcgaggtgccgtaaagcactaaatcggaaccctaaagggagcccccgatttagagcttgacggggaaagccggcgaacgtggcgagaaaggaagggaagaaagcgaaaggagcgggcgctagggcgctggcaagtgtagcggtcacgctgcgcgtaaccaccacacccgccgcgcttaatgcgccgctacagggcgcgtactatggttgctttgacgtatgcggtgtgaaataccgcacagatgcgtaaggagaaaataccgcatcaggcgccattcgccattcaggctgcgcaactgttgggaagggcgatcggtgcgggcctcttcgctattacgccagctggcgaaagggggatgtgctgcaaggcgattaagttgggtaacgccagggttttcccagtcacgacgttgtaaaacgacggccagtgaattccatggtctcaactttc

SEQ ID NO: 8 - protein, 676 aa, Dengue virus
MTAGMIIMLIPTVMAFHLTTRNGEPHMIVSRQEKGKSLLFKTKDGTNMCTLMAMDLGELCEDTITYKCPFLKQNEPEDIDCWCNSTSTWVTYGTCTTTGEHRREKRSVALVPHVGMGLETRTETWMSSEGAWKHAQRIETWILRHPGFTIMAAILAYTIGTTHFQRVLIFILLTAIAPSMTMRCIGISNRDFVEGVSGGSWVDIVLEHGSCVTTMAKNKPTLDFELIKTEAKQPATLRKYCIEAKLTNTTTDSRCPTQGEPTLNEEQDKRFVCKHSMVDRGWGNGCGLFGKGGIVTCAMFTCKKNMEGKIVQPENLEYTVVITPHSGEEHAVGNDTGKHGKEVKITPQSSITEAELTGYGTVTMECSPRTGLDFNEMVLLQMKDKAWLVHRQWFLDLPLPWLPGADTQGSNWIQKETLVTFKNPHAKKQDVVVLGSQEGAMHTALTGATEIQMSSGNLLFTGHLKCRLRMDKLQLKGMSYVMCTGSFKLEKEVAETQHGTVLVQVKYEGTDAPCKIPFSSQDEKGVTQNGRLITANPIVTDKEKPVNIEAEPPFGESYIVVGAGEKALKLSWFKKGSSIGKMFEATARGARRMAILGDTAWDFGSIGGVFTSVGKLIHQIFGTAYGVLFSGVSWTMKIGIGILLTWLGLNSRSTSLSMTCIAVGMVTLYLGVMVQA

SEQ ID NO: 9 - DNA, 6679 bp, Dengue virus
  misc_feature: Chimera DENV2 prM E (Env F108A)_chimeric DENV1 E
  CDS (906)..(2933)
  misc_feature (906)..(2336): DENV2 prM E region
  misc_feature (2337)..(2933): DENV1 region (F108A)
gaattcccattgcatacgttgtatccatatcataatatgtacatttatattggctcatgtccaacattaccgccatgttgacattgattattgactagttattaatagtaatcaattacggggtcattagttcatagcccatatatggagttccgcgttacataacttacggtaaatggcccgcctggctgaccgcccaacgacccccgcccattgacgtcaataatgacgtatgttcccatagtaacgccaatagggactttccattgacgtcaatgggtggagtatttacggtaaactgcccacttggcagtacatcaagtgtatcatatgccaagtacgccccctattgacgtcaatgacggtaaatggcccgcctggcattatgcccagtacatgaccttatgggactttcctacttggcagtacatctacgtattagtcatcgctattaccatggtgatgcggttttggcagtacatcaatgggcgtggatagcggtttgactcacggggatttccaagtctccaccccattgacgtcaatgggagtttgttttggcaccaaaatcaacgggactttccaaaatgtcgtaacaactccgccccattgacgcaaatgggcggtaggcgtgtacggtgggaggtctatataagcagagctcgtttagtgaaccgtcagatcgcctggagacgccatccacgctgttttgacctccatagaagacaccgggaccgatccagcctccgttaacggtggagggcagtgtagtctgagcagtactcgttgctgccgcgcgcgccaccagacataatagctgacagactaacagactgttcctttccatgggtcttttctgcagtcaccgtcgtcgacacgtgtgatcagatatcgcggccgccaccatgactgcaggcatgatcatcatgctgattccaacagtgatggcgtttcatctgaccacacgcaacggagaaccacacatgatcgtcagtagacaagaaaaagggaaaagccttctgtttaagacaaaggacggcacgaacatgtgtaccctcatggccatggaccttggtgagttgtgtgaagacacaatcacgtataaatgtccctttctcaagcagaacgaaccagaagacatagattgttggtgcaactccacgtccacatgggtaacttatgggacatgtaccaccacaggagagcacagaagagaaaaaagatcagtggcgcttgttccacacgtgggaatgggattggagacacgaactgaaacatggatgtcatcagaaggggcctggaaacatgcccagagaattgaaacttggattctgagacatccaggctttaccataatggccgcaatcctggcatacaccataggaacgacgcatttccaaagagtcctgatattcatcctactgacagccatcgctccttcaatgacaatgcgctgcataggaatatcaaatagggactttgtggaaggagtgtcaggagggagttgggttgacatagttttagaacatggaagttgtgtgacgacgatggcaaaaaataaaccaacactggactttgaactgataaaaacagaagccaaacaacccgccaccttaaggaagtactgtatagaggctaaactgaccaacacgacaacagactcgcgctgcccaacacaaggggaacccaccctgaatgaagagcaggacaaaaggtttgtctgcaaacattccatggtagacagaggatggggaaatggatgtggattagctggaaaaggaggcatcgtgacctgtgccatgttcacatgcaaaaagaacatggagggaaaaattgtgcagccagaaaacctggaatacactgtcgttataacacctcattcaggggaagaacatgcagtcggaaatgacacaggaaaacatggtaaagaagtcaagataacaccacagagctccatcacagaggcggaactgacaggctatggcactgttacgatggagtgctctccaagaacgggcctcgacttcaatgagatggtgttgctgcaaatgaaagacaaagcttggctggtgcacagacaatggttcctagacctaccgttgccatggctgcccggagcagacacacaaggatcaaattggatacagaaagagacactggtcaccttcaaaaatccccatgcgaaaaaacaggatgttgttgtcttaggctcccaagagggggccatgcatacagcactcacaggggctacggaaatccagatgtcatcaggaaacctgctgttcacaggacatcttaagtgcaggctgagaatggacaaattacaacttaaagggatgtcatatgtaatgtgcacagggtcattcaagttagagaaggaagtggctgagacccagcatggaactgttctagtgcaggttaaatacgaaggaacagatgcaccatgcaagatccccttctcgtcccaagatgagaagggagtaacccagaatgggagattgataacagccaaccccatagtcactgacaaagaaaaaccagtcaacattgaagcggagccaccttttggtgagagctacattgtggtaggagcaggtgaaaaagctttgaaactaagctggttcaagaagggaagcagtatagggaaaatgtttgaagcaactgcccgtggagcacgaaggatggccatcctgggagacactgcatgggacttcggttctataggaggggtgttcacgtctgtgggaaaactgatacaccagatttttgggactgcgtatggagttttgttcagcggtgtttcttggaccatgaagataggaatagggattctgctgacatggctaggattaaactcaaggagcacgtccctttcaatgacgtgtatcgcagttggcatggtcacgctgtacctaggagtcatggttcaggcgtaataaagatctgctgtgccttctagttgccagccatctgttgtttgcccctcccccgtgccttccttgaccctggaaggtgccactcccactgtcctttcctaataaaatgaggaaattgcatcgcattgtctgagtaggtgtcattctattctggggggtggggtggggcaggacagcaagggggaggattgggaagacaatagcaggcatgctggggatgcggtgggctctatgggtacccaggtgctgaagaattgacccggttcctcctgggccagaaagaagcaggcacatccccttctctgtgacacaccctgtccacgcccctggttcttagttccagccccactcataggacactcatagctcaggagggctccgccttcaatcccacccgctaaagtacttggagcggtctctccctccctcatcagcccaccaaaccaaacctagcctccaagagtgggaagaaattaaagcaagataggctattaagtgcagagggagagaaaatgcctccaacatgtgaggaagtaatgagagaaatcatagaattttaaggccatgatttaaggccatcatggcctaagcttgaaaggagataggatcaaagcttggcgtaatcatggtcatagctgtttcctgtgtgaaattgttatccgctcacaattccacacaacatacgagccggaagcataaagtgtaaagcctggggtgcctaatgagtgagctaactcacattaattgcgttgcgctcactgcccgctttccagtcgggaaacctgtcgtgccagctgcattaatgaatcggccaacgcgcggggagaggcggtttgcgtattgggcgctcttccgcttcctcgctcactgactcgctgcgctcggtcgttcggctgcggcgagcggtatcagctcactcaaaggcggtaatacggttatccacagaatcaggggataacgcaggaaagaacatgtgagcaaaaggccagcaaaaggccaggaaccgtaaaaaggccgcgttgctggcgtttttccataggctccgcccccctgacgagcatcacaaaaatcgacgctcaagtcagaggtggcgaaacccgacaggactataaagataccaggcgtttccccctggaagctccctcgtgcgctctcctgttccgaccctgccgcttaccggatacctgtccgcctttctcccttcgggaagcgtggcgctttctcatagctcacgctgtaggtatctcagttcggtgtaggtcgttcgctccaagctgggctgtgtgcacgaaccccccgttcagcccgaccgctgcgccttatccggtaactatcgtcttgagtccaacccggtaagacacgacttatcgccactggcagcagccactggtaacaggattagcagagcgaggtatgtaggcggtgctacagagttcttgaagtggtggcctaactacggctacactagaagaacagtatttggtatctgcgctctgctgaagccagttaccttcggaaaaagagttggtagctcttgatccggcaaacaaaccaccgctggtagcggtggtttttttgtttgcaagcagcagattacgcgcagaaaaaaaggatctcaagaagatcctttgatcttttctacggggtctgacgctcagtggaacgaaaactcacgttaagggattttggtcatgagattatcaaaaaggatcttcacctagatccttttaaattaaaaatgaagttttaaatcaatctaaagtatatatgagtaaacttggtctgacagttaccaatgcttaatcagtgaggcacctatctcagcgatctgtctatttcgttcatccatagttgcctgactccccgtcgtgtagataactacgatacgggagggcttaccatctggccccagtgctgcaatgataccgcgagaaccacgctcaccggctccagatttatcagcaataaaccagccagccggaagggccgagcgcagaagtggtcctgcaactttatccgcctccatccagtctattaattgttgccgggaagctagagtaagtagttcgccagttaatagtttgcgcaacgttgttgccattgctacaggcatcgtggtgtcacgctcgtcgtttggtatggcttcattcagctccggttcccaacgatcaaggcgagttacatgatcccccatgttgtgcaaaaaagcggttagctccttcggtcctccgatcgttgtcagaagtaagttggccgcagtgttatcactcatggttatggcagcactgcataattctcttactgtcatgccatccgtaagatgcttttctgtgactggtgagtactcaaccaagtcattctgagaatagtgtatgcggcgaccgagttgctcttgcccggcgtcaatacgggataataccgcgccacatagcagaactttaaaagtgctcatcattggaaaacgttcttcggggcgaaaactctcaaggatcttaccgctgttgagatccagttcgatgtaacccactcgtgcacccaactgatcttcagcatcttttactttcaccagcgtttctgggtgagcaaaaacaggaaggcaaaatgccgcaaaaaagggaataagggcgacacggaaatgttgaatactcatactcttcctttttcaatattattgaagcatttatcagggttattgtctcatgagcggatacatatttgaatgtatttagaaaaataaacaaataggggttccgcgcacatttccccgaaaagtgccacctgacgtctaagaaaccattattatcatgacattaacctataaaaataggcgtatcacgaggccctttcgggtcgcgcgtttcggtgatgacggtgaaaacctctgacacatgcagctcccgttgacggtcacagcttgtctgtaagcggatgccgggagcagacaagcccgtcagggcgcgtcagcgggtgttggcgggtgtcggggctggcttaactatgcggcatcagagcagattgtactgagagtgcaccataaaattgtaaacgttaatattttgttaaaattcgcgttaaatttttgttaaatcagctcattttttaaccaataggccgaaatcggcaaaatcccttataaatcaaaagaatagcccgagatagggttgagtgttgttccagtttggaacaagagtccactattaaagaacgtggactccaacgtcaaagggcgaaaaaccgtctatcagggcgatggcccactacgtgaaccatcacccaaatcaagttttttggggtcgaggtgccgtaaagcactaaatcggaaccctaaagggagcccccgatttagagcttgacggggaaagccggcgaacgtggcgagaaaggaagggaagaaagcgaaaggagcgggcgctagggcgctggcaagtgtagcggtcacgctgcgcgtaaccaccacacccgccgcgcttaatgcgccgctacagggcgcgtactatggttgctttgacgtatgcggtgtgaaataccgcacagatgcgtaaggagaaaataccgcatcaggcgccattcgccattcaggctgcgcaactgttgggaagggcgatcggtgcgggcctcttcgctattacgccagctggcgaaagggggatgtgctgcaaggcgattaagttgggtaacgccagggttttcccagtcacgacgttgtaaaacgacggccagtgaattccatggtctcaactttc

SEQ ID NO: 10 - protein, 676 aa, Dengue virus
MTAGMIIMLIPTVMAFHLTTRNGEPHMIVSRQEKGKSLLFKTKDGTNMCTLMAMDLGELCEDTITYKCPFLKQNEPEDIDCWCNSTSTWVTYGTCTTTGEHRREKRSVALVPHVGMGLETRTETWMSSEGAWKHAQRIETWILRHPGFTIMAAILAYTIGTTHFQRVLIFILLTAIAPSMTMRCIGISNRDFVEGVSGGSWVDIVLEHGSCVTTMAKNKPTLDFELIKTEAKQPATLRKYCIEAKLTNTTTDSRCPTQGEPTLNEEQDKRFVCKHSMVDRGWGNGCGLAGKGGIVTCAMFTCKKNMEGKIVQPENLEYTVVITPHSGEEHAVGNDTGKHGKEVKITPQSSITEAELTGYGTVTMECSPRTGLDFNEMVLLQMKDKAWLVHRQWFLDLPLPWLPGADTQGSNWIQKETLVTFKNPHAKKQDVVVLGSQEGAMHTALTGATEIQMSSGNLLFTGHLKCRLRMDKLQLKGMSYVMCTGSFKLEKEVAETQHGTVLVQVKYEGTDAPCKIPFSSQDEKGVTQNGRLITANPIVTDKEKPVNIEAEPPFGESYIVVGAGEKALKLSWFKKGSSIGKMFEATARGARRMAILGDTAWDFGSIGGVFTSVGKLIHQIFGTAYGVLFSGVSWTMKIGIGILLTWLGLNSRSTSLSMTCIAVGMVTLYLGVMVQA

SEQ ID NO: 11 - DNA, 3770 bp, Dengue virus
  misc_feature: DENV2 capsid R85A K86A mutant
  CDS (1046)..(1345)
tcgcgcgtttcggtgatgacggtgaaaacctctgacacatgcagctcccggagacggtcacagcttgtctgtaagcggatgccgggagcagacaagcccgtcagggcgcgtcagcgggtgttggcgggtgtcggggctggcttaactatgcggcatcagagcagattgtactgagagtgcaccatatgcggtgtgaaataccgcacagatgcgtaaggagaaaataccgcatcaggcgccattcgccattcaggctgcgcaactgttgggaagggcgatcggtgcgggcctcttcgctattacgccagctggcgaaagggggatgtgctgcaaggcgattaagttgggtaacgccagggttttcccagtcacgacgttgtaaaacgacggccagtgaattgacgcgtttgacattgattattgactagttattaatagtaatcaattacggggtcattagttcatagcccatatatggagttccgcgttacataacttacggtaaatggcccgcctggctgaccgcccaacgacccccgcccattgacgtcaataatgacgtatgttcccatagtaacgccaatagggactttccattgacgtcaatgggtggagtatttacggtaaactgcccacttggcagtacatcaagtgtatcatatgccaagtacgccccctattgacgtcaatgacggtaaatggcccgcctggcattatgcccagtacatgaccttatgggactttcctacttggcagtacatctacgtattagtcatcgctattaccatggtgatgcggttttggcagtacatcaatgggcgtggatagcggtttgactcacggggatttccaagtctccaccccattgacgtcaatgggagtttgttttggcaccaaaatcaacgggactttccaaaatgtcgtaacaactccgccccattgacgcaaatgggcggtaggcgtgtacggtgggaggtctatataagcagagctcgtttagtgaaccgtcagataactgcaggtcgacgatatcgcggccgccaccatgaatgaccaacggaaaaaggcgagaaacacgcctttcaatatgctgaaacgcgagagaaaccgcgtgtcaactgtacaacagttgacaaagagattctcacttggaatgctgcagggacgaggaccactaaaattgttcatggccctggtggcattccttcgtttcctaacaatcccaccaacagcagggatattaaaaagatggggaacaattaaaaaatcaaaggctattaatgttctgagaggcttcgcggcagagattggaaggatgctgaatatcttaaacaggagacgtagataataaagatctgctgtgccttctagttgccagccatctgttgtttgcccctcccccgtgccttccttgaccctggaaggtgccactcccactgtcctttcctaataaaatgaggaaattgcatcgcattgtctgagtaggtgtcattctattctggggggtggggtggggcaggacagcaagggggaggattgggaagacaatagcaggcatgctggggatgcggtgggctctatggctcgagcatggtcatagctgtttcctgtgtgaaattgttatccgctcacaattccacacaacatacgagccggaagcataaagtgtaaagcctggggtgcctaatgagtgagctaactcacattaattgcgttgcgctcactgcccgctttccagtcgggaaacctgtcgtgccagctgcattaatgaatcggccaacgcgcggggagaggcggtttgcgtattgggcgctcttccgcttcctcgctcactgactcgctgcgctcggtcgttcggctgcggcgagcggtatcagctcactcaaaggcggtaatacggttatccacagaatcaggggataacgcaggaaagaacatgtgagcaaaaggccagcaaaaggccaggaaccgtaaaaaggccgcgttgctggcgtttttccataggctccgcccccctgacgagcatcacaaaaatcgacgctcaagtcagaggtggcgaaacccgacaggactataaagataccaggcgtttccccctggaagctccctcgtgcgctctcctgttccgaccctgccgcttaccggatacctgtccgcctttctcccttcgggaagcgtggcgctttctcatagctcacgctgtaggtatctcagttcggtgtaggtcgttcgctccaagctgggctgtgtgcacgaaccccccgttcagcccgaccgctgcgccttatccggtaactatcgtcttgagtccaacccggtaagacacgacttatcgccactggcagcagccactggtaacaggattagcagagcgaggtatgtaggcggtgctacagagttcttgaagtggtggcctaactacggctacactagaagaacagtatttggtatctgcgctctgctgaagccagttaccttcggaaaaagagttggtagctcttgatccggcaaacaaaccaccgctggtagcggtggtttttttgtttgcaagcagcagattacgcgcagaaaaaaaggatctcaagaagatcctttgatcttttctacggggtctgacgctcagtggaacgaaaactcacgttaagggattttggtcatgagattatcaaaaaggatcttcacctagatccttttaaattaaaaatgaagttttaaatcaatctaaagtatatatgagtaaacttggtctgacagttagaaaaactcatcgagcatcaaatgaaactgcaatttattcatatcaggattatcaataccatatttttgaaaaagccgtttctgtaatgaaggagaaaactcaccgaggcagttccataggatggcaagatcctggtatcggtctgcgattccgactcgtccaacatcaatacaacctattaatttcccctcgtcaaaaataaggttatcaagtgagaaatcaccatgagtgacgactgaatccggtgagaatggcaaaagtttatgcatttctttccagacttgttcaacaggccagccattacgctcgtcatcaaaatcactcgcatcaaccaaaccgttattcattcgtgattgcgcctgagcgagacgaaatacgcgatcgctgttaaaaggacaattacaaacaggaatcgaatgcaaccggcgcaggaacactgccagcgcatcaacaatattttcacctgaatcaggatattcttctaatacctggaatgctgttttcccagggatcgcagtggtgagtaaccatgcatcatcaggagtacggataaaatgcttgatggtcggaagaggcataaattccgtcagccagtttagtctgaccatctcatctgtaacatcattggcaacgctacctttgccatgtttcagaaacaactctggcgcatcgggcttcccatacaatcgatagattgtcgcacctgattgcccgacattatcgcgagcccatttatacccatataaatcagcatccatgttggaatttaatcgcggcctagagcaagacgtttcccgttgaatatggctcatactcttcctttttcaatattattgaagcatttatcagggttattgtctcatgagcggatacatatttgaatgtatttagaaaaataaacaaataggggttccgcgcacatttccccgaaaagtgccacctgacgtctaagaaaccattattatcatgacattaacctataaaaataggcgtatcacgaggccctttcgtc

SEQ ID NO: 12 - protein, 100 aa, Dengue virus
MNDQRKKARNTPFNMLKRERNRVSTVQQLTKRFSLGMLQGRGPLKLFMALVAFLRFLTIPPTAGILKRWGTIKKSKAINVLRGFAAEIGRMLNILNRRRR

SEQ ID NO: 13 - DNA, 6910 bp, Dengue virus
  misc_feature: DENV1 prM E (F108A K246M)
  CDS (1137)..(3164)
gaattcccattgcatacgttgtatccatatcataatatgtacatttatattggctcatgtccaacattaccgccatgttgacattgattattgactagttattaatagtaatcaattacggggtcattagttcatagcccatatatggagttccgcgttacataacttacggtaaatggcccgcctggctgaccgcccaacgacccccgcccattgacgtcaataatgacgtatgttcccatagtaacgccaatagggactttccattgacgtcaatgggtggagtatttacggtaaactgcccacttggcagtacatcaagtgtatcatatgccaagtacgccccctattgacgtcaatgacggtaaatggcccgcctggcattatgcccagtacatgaccttatgggactttcctacttggcagtacatctacgtattagtcatcgctattaccatggtgatgcggttttggcagtacatcaatgggcgtggatagcggtttgactcacggggatttccaagtctccaccccattgacgtcaatgggagtttgttttggcaccaaaatcaacgggactttccaaaatgtcgtaacaactccgccccattgacgcaaatgggcggtaggcgtgtacggtgggaggtctatataagcagagctcgtttagtgaaccgtcagatcgcctggagacgccatccacgctgttttgacctccatagaagacaccgggaccgatccagcctccatcggctcgcatctctccttcacgcgcccgccgccctacctgaggccgccatccacgccggttgagtcgcgttctgccgcctcccgcctgtggtgcctcctgaactgcgtccgccgtctaggtaagtttaaagctcaggtcgagaccgggcctttgtccggcgctcccttggagcctacctagactcagccggctctccacgctttgcctgaccctgcttgctcaactctagttaacggtggagggcagtgtagtctgagcagtactcgttgctgccgcgcgcgccaccagacataatagctgacagactaacagactgttcctttccatgggtcttttctgcagtcaccgtcgtcgacacgtgtgatcagatatcgcggccgccaccatgtcggtgaccatgctcctcatgctgctgcccacagccctggcgttccatctgaccacccgagggggagagccgcacatgatagttagcaagcaggaaagaggaaaatcacttttgtttaagacctctgcaggtgtcaacatgtgcacccttattgcaatggatttgggagagttatgtgaggacacaatgacctacaaatgcccccggatcactgagacggaaccagatgacgttgactgttggtgcaatgccacggagacatgggtgacctatggaacatgttctcaaactggtgaacaccgacgagacaaacgttccgtcgcactggcaccacacgtagggcttggtctagaaacaagaaccgaaacgtggatgtcctctgaaggcgcttggaaacaaatacaaaaagtggagacctgggctctgagacacccaggattcacggtgatagccctttttctagcacatgccataggaacatccatcacccagaaagggatcatttttattttgctgatgctggtaactccatccatggccatgcggtgcgtgggaataggcaacagagacttcgtggaaggactgtcaggagctacgtgggtggatgtggtactggagcatggaagttgcgtcactaccatggcaaaagacaaaccaacactggacattgaactcttgaagacggaggtcacaaaccctgccgtcctgcgcaaactgtgcattgaagctaaaatatcaaacaccaccaccgattcgagatgtccaacacaaggagaagccacgctggtggaagaacaggacacgaactttgtgtgtcgacgaacgttcgtggacagaggctggggcaatggttgtgggctagccggaaaaggtagcttaataacgtgtgctaagtttaagtgtgtgacaaaactggaaggaaagatagtccaatatgaaaacttaaaatattcagtgatagtcaccgtacacactggagaccagcaccaagttggaaatgagaccacagaacatggaacaactgcaaccataacacctcaagctcccacgtcggaaatacagctgacagactacggagctctaacattggattgttcacctagaacagggctagactttaatgagatggtgttgttgacaatggaaaataaatcatggctcgtccacaaacaatggtttctagacttaccactgccttggacctcgggggcttcaacatcccaagagacttggaatagacaagacttgctggtcacatttaagacagctcatgcaaaaaagcaggaagtagtcgtactaggatcacaagaaggagcaatgcacactgcgttgactggagcgacagaaatccaaacgtctggaacgacaacaatttttgcaggacacctgaaatgcagactaaaaatggataaactgactttaaaagggatgtcatatgtaatgtgcacagggtcattcaagttagagaaggaagtggctgagacccagcatggaactgttctagtgcaggttaaatacgaaggaacagatgcaccatgcaagatccccttctcgtcccaagatgagaagggagtaacccagaatgggagattgataacagccaaccccatagtcactgacaaagaaaaaccagtcaacattgaagcggagccaccttttggtgagagctacattgtggtaggagcaggtgaaaaagctttgaaactaagctggttcaagaagggaagcagtatagggaaaatgtttgaagcaactgcccgtggagcacgaaggatggccatcctgggagacactgcatgggacttcggttctataggaggggtgttcacgtctgtgggaaaactgatacaccagatttttgggactgcgtatggagttttgttcagcggtgtttcttggaccatgaagataggaatagggattctgctgacatggctaggattaaactcaaggagcacgtccctttcaatgacgtgtatcgcagttggcatggtcacgctgtacctaggagtcatggttcaggcgtaataaagatctgctgtgccttctagttgccagccatctgttgtttgcccctcccccgtgccttccttgaccctggaaggtgccactcccactgtcctttcctaataaaatgaggaaattgcatcgcattgtctgagtaggtgtcattctattctggggggtggggtggggcaggacagcaagggggaggattgggaagacaatagcaggcatgctggggatgcggtgggctctatgggtacccaggtgctgaagaattgacccggttcctcctgggccagaaagaagcaggcacatccccttctctgtgacacaccctgtccacgcccctggttcttagttccagccccactcataggacactcatagctcaggagggctccgccttcaatcccacccgctaaagtacttggagcggtctctccctccctcatcagcccaccaaaccaaacctagcctccaagagtgggaagaaattaaagcaagataggctattaagtgcagagggagagaaaatgcctccaacatgtgaggaagtaatgagagaaatcatagaattttaaggccatgatttaaggccatcatggcctaagcttgaaaggagataggatcaaagcttggcgtaatcatggtcatagctgtttcctgtgtgaaattgttatccgctcacaattccacacaacatacgagccggaagcataaagtgtaaagcctggggtgcctaatgagtgagctaactcacattaattgcgttgcgctcactgcccgctttccagtcgggaaacctgtcgtgccagctgcattaatgaatcggccaacgcgcggggagaggcggtttgcgtattgggcgctcttccgcttcctcgctcactgactcgctgcgctcggtcgttcggctgcggcgagcggtatcagctcactcaaaggcggtaatacggttatccacagaatcaggggataacgcaggaaagaacatgtgagcaaaaggccagcaaaaggccaggaaccgtaaaaaggccgcgttgctggcgtttttccataggctccgcccccctgacgagcatcacaaaaatcgacgctcaagtcagaggtggcgaaacccgacaggactataaagataccaggcgtttccccctggaagctccctcgtgcgctctcctgttccgaccctgccgcttaccggatacctgtccgcctttctcccttcgggaagcgtggcgctttctcatagctcacgctgtaggtatctcagttcggtgtaggtcgttcgctccaagctgggctgtgtgcacgaaccccccgttcagcccgaccgctgcgccttatccggtaactatcgtcttgagtccaacccggtaagacacgacttatcgccactggcagcagccactggtaacaggattagcagagcgaggtatgtaggcggtgctacagagttcttgaagtggtggcctaactacggctacactagaagaacagtatttggtatctgcgctctgctgaagccagttaccttcggaaaaagagttggtagctcttgatccggcaaacaaaccaccgctggtagcggtggtttttttgtttgcaagcagcagattacgcgcagaaaaaaaggatctcaagaagatcctttgatcttttctacggggtctgacgctcagtggaacgaaaactcacgttaagggattttggtcatgagattatcaaaaaggatcttcacctagatccttttaaattaaaaatgaagttttaaatcaatctaaagtatatatgagtaaacttggtctgacagttaccaatgcttaatcagtgaggcacctatctcagcgatctgtctatttcgttcatccatagttgcctgactccccgtcgtgtagataactacgatacgggagggcttaccatctggccccagtgctgcaatgataccgcgagaaccacgctcaccggctccagatttatcagcaataaaccagccagccggaagggccgagcgcagaagtggtcctgcaactttatccgcctccatccagtctattaattgttgccgggaagctagagtaagtagttcgccagttaatagtttgcgcaacgttgttgccattgctacaggcatcgtggtgtcacgctcgtcgtttggtatggcttcattcagctccggttcccaacgatcaaggcgagttacatgatcccccatgttgtgcaaaaaagcggttagctccttcggtcctccgatcgttgtcagaagtaagttggccgcagtgttatcactcatggttatggcagcactgcataattctcttactgtcatgccatccgtaagatgcttttctgtgactggtgagtactcaaccaagtcattctgagaatagtgtatgcggcgaccgagttgctcttgcccggcgtcaatacgggataataccgcgccacatagcagaactttaaaagtgctcatcattggaaaacgttcttcggggcgaaaactctcaaggatcttaccgctgttgagatccagttcgatgtaacccactcgtgcacccaactgatcttcagcatcttttactttcaccagcgtttctgggtgagcaaaaacaggaaggcaaaatgccgcaaaaaagggaataagggcgacacggaaatgttgaatactcatactcttcctttttcaatattattgaagcatttatcagggttattgtctcatgagcggatacatatttgaatgtatttagaaaaataaacaaataggggttccgcgcacatttccccgaaaagtgccacctgacgtctaagaaaccattattatcatgacattaacctataaaaataggcgtatcacgaggccctttcgggtcgcgcgtttcggtgatgacggtgaaaacctctgacacatgcagctcccgttgacggtcacagcttgtctgtaagcggatgccgggagcagacaagcccgtcagggcgcgtcagcgggtgttggcgggtgtcggggctggcttaactatgcggcatcagagcagattgtactgagagtgcaccataaaattgtaaacgttaatattttgttaaaattcgcgttaaatttttgttaaatcagctcattttttaaccaataggccgaaatcggcaaaatcccttataaatcaaaagaatagcccgagatagggttgagtgttgttccagtttggaacaagagtccactattaaagaacgtggactccaacgtcaaagggcgaaaaaccgtctatcagggcgatggcccactacgtgaaccatcacccaaatcaagttttttggggtcgaggtgccgtaaagcactaaatcggaaccctaaagggagcccccgatttagagcttgacggggaaagccggcgaacgtggcgagaaaggaagggaagaaagcgaaaggagcgggcgctagggcgctggcaagtgtagcggtcacgctgcgcgtaaccaccacacccgccgcgcttaatgcgccgctacagggcgcgtactatggttgctttgacgtatgcggtgtgaaataccgcacagatgcgtaaggagaaaataccgcatcaggcgccattcgccattcaggctgcgcaactgttgggaagggcgatcggtgcgggcctcttcgctattacgccagctggcgaaagggggatgtgctgcaaggcgattaagttgggtaacgccagggttttcccagtcacgacgttgtaaaacgacggccagtgaattccatggtctcaactttc

SEQ ID NO: 14 - protein, 676 aa, Dengue virus
MSVTMLLMLLPTALAFHLTTRGGEPHMIVSKQERGKSLLFKTSAGVNMCTLIAMDLGELCEDTMTYKCPRITETEPDDVDCWCNATETWVTYGTCSQTGEHRRDKRSVALAPHVGLGLETRTETWMSSEGAWKQIQKVETWALRHPGFTVIALFLAHAIGTSITQKGIIFILLMLVTPSMAMRCVGIGNRDFVEGLSGATWVDVVLEHGSCVTTMAKDKPTLDIELLKTEVTNPAVLRKLCIEAKISNTTTDSRCPTQGEATLVEEQDTNFVCRRTFVDRGWGNGCGLAGKGSLITCAKFKCVTKLEGKIVQYENLKYSVIVTVHTGDQHQVGNETTEHGTTATITPQAPTSEIQLTDYGALTLDCSPRTGLDFNEMVLLTMENKSWLVHKQWFLDLPLPWTSGASTSQETWNRQDLLVTFKTAHAKKQEVVVLGSQEGAMHTALTGATEIQTSGTTTIFAGHLKCRLKMDKLTLKGMSYVMCTGSFKLEKEVAETQHGTVLVQVKYEGTDAPCKIPFSSQDEKGVTQNGRLITANPIVTDKEKPVNIEAEPPFGESYIVVGAGEKALKLSWFKKGSSIGKMFEATARGARRMAILGDTAWDFGSIGGVFTSVGKLIHQIFGTAYGVLFSGVSWTMKIGIGILLTWLGLNSRSTSLSMTCIAVGMVTLYLGVMVQA

SEQ ID NO: 15 - DNA, 6910 bp, Dengue virus
  misc_feature: DENV1 prM E (F108A K203N) VLP D01
  CDS (1137)..(3164)
gaattcccattgcatacgttgtatccatatcataatatgtacatttatattggctcatgtccaacattaccgccatgttgacattgattattgactagttattaatagtaatcaattacggggtcattagttcatagcccatatatggagttccgcgttacataacttacggtaaatggcccgcctggctgaccgcccaacgacccccgcccattgacgtcaataatgacgtatgttcccatagtaacgccaatagggactttccattgacgtcaatgggtggagtatttacggtaaactgcccacttggcagtacatcaagtgtatcatatgccaagtacgccccctattgacgtcaatgacggtaaatggcccgcctggcattatgcccagtacatgaccttatgggactttcctacttggcagtacatctacgtattagtcatcgctattaccatggtgatgcggttttggcagtacatcaatgggcgtggatagcggtttgactcacggggatttccaagtctccaccccattgacgtcaatgggagtttgttttggcaccaaaatcaacgggactttccaaaatgtcgtaacaactccgccccattgacgcaaatgggcggtaggcgtgtacggtgggaggtctatataagcagagctcgtttagtgaaccgtcagatcgcctggagacgccatccacgctgttttgacctccatagaagacaccgggaccgatccagcctccatcggctcgcatctctccttcacgcgcccgccgccctacctgaggccgccatccacgccggttgagtcgcgttctgccgcctcccgcctgtggtgcctcctgaactgcgtccgccgtctaggtaagtttaaagctcaggtcgagaccgggcctttgtccggcgctcccttggagcctacctagactcagccggctctccacgctttgcctgaccctgcttgctcaactctagttaacggtggagggcagtgtagtctgagcagtactcgttgctgccgcgcgcgccaccagacataatagctgacagactaacagactgttcctttccatgggtcttttctgcagtcaccgtcgtcgacacgtgtgatcagatatcgcggccgccaccatgtcggtgaccatgctcctcatgctgctgcccacagccctggcgttccatctgaccacccgagggggagagccgcacatgatagttagcaagcaggaaagaggaaaatcacttttgtttaagacctctgcaggtgtcaacatgtgcacccttattgcaatggatttgggagagttatgtgaggacacaatgacctacaaatgcccccggatcactgagacggaaccagatgacgttgactgttggtgcaatgccacggagacatgggtgacctatggaacatgttctcaaactggtgaacaccgacgagacaaacgttccgtcgcactggcaccacacgtagggcttggtctagaaacaagaaccgaaacgtggatgtcctctgaaggcgcttggaaacaaatacaaaaagtggagacctgggctctgagacacccaggattcacggtgatagccctttttctagcacatgccataggaacatccatcacccagaaagggatcatttttattttgctgatgctggtaactccatccatggccatgcggtgcgtgggaataggcaacagagacttcgtggaaggactgtcaggagctacgtgggtggatgtggtactggagcatggaagttgcgtcactaccatggcaaaagacaaaccaacactggacattgaactcttgaagacggaggtcacaaaccctgccgtcctgcgcaaactgtgcattgaagctaaaatatcaaacaccaccaccgattcgagatgtccaacacaaggagaagccacgctggtggaagaacaggacacgaactttgtgtgtcgacgaacgttcgtggacagaggctggggcaatggttgtgggctagccggaaaaggtagcttaataacgtgtgctaagtttaagtgtgtgacaaaactggaaggaaagatagtccaatatgaaaacttaaaatattcagtgatagtcaccgtacacactggagaccagcaccaagttggaaatgagaccacagaacatggaacaactgcaaccataacacctcaagctcccacgtcggaaatacagctgacagactacggagctctaacattggattgttcacctagaacagggctagactttaatgagatggtgttgttgacaatggaaaaaaaatcatggctcgtccacaaacaatggtttctagacttaccactgccttggacctcgggggcttcaacatcccaagagacttggaatagacaagacttgctggtcacatttaagacagctcatgcaatgaagcaggaagtagtcgtactaggatcacaagaaggagcaatgcacactgcgttgactggagcgacagaaatccaaacgtctggaacgacaacaatttttgcaggacacctgaaatgcagactaaaaatggataaactgactttaaaagggatgtcatatgtaatgtgcacagggtcattcaagttagagaaggaagtggctgagacccagcatggaactgttctagtgcaggttaaatacgaaggaacagatgcaccatgcaagatccccttctcgtcccaagatgagaagggagtaacccagaatgggagattgataacagccaaccccatagtcactgacaaagaaaaaccagtcaacattgaagcggagccaccttttggtgagagctacattgtggtaggagcaggtgaaaaagctttgaaactaagctggttcaagaagggaagcagtatagggaaaatgtttgaagcaactgcccgtggagcacgaaggatggccatcctgggagacactgcatgggacttcggttctataggaggggtgttcacgtctgtgggaaaactgatacaccagatttttgggactgcgtatggagttttgttcagcggtgtttcttggaccatgaagataggaatagggattctgctgacatggctaggattaaactcaaggagcacgtccctttcaatgacgtgtatcgcagttggcatggtcacgctgtacctaggagtcatggttcaggcgtaataaagatctgctgtgccttctagttgccagccatctgttgtttgcccctcccccgtgccttccttgaccctggaaggtgccactcccactgtcctttcctaataaaatgaggaaattgcatcgcattgtctgagtaggtgtcattctattctggggggtggggtggggcaggacagcaagggggaggattgggaagacaatagcaggcatgctggggatgcggtgggctctatgggtacccaggtgctgaagaattgacccggttcctcctgggccagaaagaagcaggcacatccccttctctgtgacacaccctgtccacgcccctggttcttagttccagccccactcataggacactcatagctcaggagggctccgccttcaatcccacccgctaaagtacttggagcggtctctccctccctcatcagcccaccaaaccaaacctagcctccaagagtgggaagaaattaaagcaagataggctattaagtgcagagggagagaaaatgcctccaacatgtgaggaagtaatgagagaaatcatagaattttaaggccatgatttaaggccatcatggcctaagcttgaaaggagataggatcaaagcttggcgtaatcatggtcatagctgtttcctgtgtgaaattgttatccgctcacaattccacacaacatacgagccggaagcataaagtgtaaagcctggggtgcctaatgagtgagctaactcacattaattgcgttgcgctcactgcccgctttccagtcgggaaacctgtcgtgccagctgcattaatgaatcggccaacgcgcggggagaggcggtttgcgtattgggcgctcttccgcttcctcgctcactgactcgctgcgctcggtcgttcggctgcggcgagcggtatcagctcactcaaaggcggtaatacggttatccacagaatcaggggataacgcaggaaagaacatgtgagcaaaaggccagcaaaaggccaggaaccgtaaaaaggccgcgttgctggcgtttttccataggctccgcccccctgacgagcatcacaaaaatcgacgctcaagtcagaggtggcgaaacccgacaggactataaagataccaggcgtttccccctggaagctccctcgtgcgctctcctgttccgaccctgccgcttaccggatacctgtccgcctttctcccttcgggaagcgtggcgctttctcatagctcacgctgtaggtatctcagttcggtgtaggtcgttcgctccaagctgggctgtgtgcacgaaccccccgttcagcccgaccgctgcgccttatccggtaactatcgtcttgagtccaacccggtaagacacgacttatcgccactggcagcagccactggtaacaggattagcagagcgaggtatgtaggcggtgctacagagttcttgaagtggtggcctaactacggctacactagaagaacagtatttggtatctgcgctctgctgaagccagttaccttcggaaaaagagttggtagctcttgatccggcaaacaaaccaccgctggtagcggtggtttttttgtttgcaagcagcagattacgcgcagaaaaaaaggatctcaagaagatcctttgatcttttctacggggtctgacgctcagtggaacgaaaactcacgttaagggattttggtcatgagattatcaaaaaggatcttcacctagatccttttaaattaaaaatgaagttttaaatcaatctaaagtatatatgagtaaacttggtctgacagttaccaatgcttaatcagtgaggcacctatctcagcgatctgtctatttcgttcatccatagttgcctgactccccgtcgtgtagataactacgatacgggagggcttaccatctggccccagtgctgcaatgataccgcgagaaccacgctcaccggctccagatttatcagcaataaaccagccagccggaagggccgagcgcagaagtggtcctgcaactttatccgcctccatccagtctattaattgttgccgggaagctagagtaagtagttcgccagttaatagtttgcgcaacgttgttgccattgctacaggcatcgtggtgtcacgctcgtcgtttggtatggcttcattcagctccggttcccaacgatcaaggcgagttacatgatcccccatgttgtgcaaaaaagcggttagctccttcggtcctccgatcgttgtcagaagtaagttggccgcagtgttatcactcatggttatggcagcactgcataattctcttactgtcatgccatccgtaagatgcttttctgtgactggtgagtactcaaccaagtcattctgagaatagtgtatgcggcgaccgagttgctcttgcccggcgtcaatacgggataataccgcgccacatagcagaactttaaaagtgctcatcattggaaaacgttcttcggggcgaaaactctcaaggatcttaccgctgttgagatccagttcgatgtaacccactcgtgcacccaactgatcttcagcatcttttactttcaccagcgtttctgggtgagcaaaaacaggaaggcaaaatgccgcaaaaaagggaataagggcgacacggaaatgttgaatactcatactcttcctttttcaatattattgaagcatttatcagggttattgtctcatgagcggatacatatttgaatgtatttagaaaaataaacaaataggggttccgcgcacatttccccgaaaagtgccacctgacgtctaagaaaccattattatcatgacattaacctataaaaataggcgtatcacgaggccctttcgggtcgcgcgtttcggtgatgacggtgaaaacctctgacacatgcagctcccgttgacggtcacagcttgtctgtaagcggatgccgggagcagacaagcccgtcagggcgcgtcagcgggtgttggcgggtgtcggggctggcttaactatgcggcatcagagcagattgtactgagagtgcaccataaaattgtaaacgttaatattttgttaaaattcgcgttaaatttttgttaaatcagctcattttttaaccaataggccgaaatcggcaaaatcccttataaatcaaaagaatagcccgagatagggttgagtgttgttccagtttggaacaagagtccactattaaagaacgtggactccaacgtcaaagggcgaaaaaccgtctatcagggcgatggcccactacgtgaaccatcacccaaatcaagttttttggggtcgaggtgccgtaaagcactaaatcggaaccctaaagggagcccccgatttagagcttgacggggaaagccggcgaacgtggcgagaaaggaagggaagaaagcgaaaggagcgggcgctagggcgctggcaagtgtagcggtcacgctgcgcgtaaccaccacacccgccgcgcttaatgcgccgctacagggcgcgtactatggttgctttgacgtatgcggtgtgaaataccgcacagatgcgtaaggagaaaataccgcatcaggcgccattcgccattcaggctgcgcaactgttgggaagggcgatcggtgcgggcctcttcgctattacgccagctggcgaaagggggatgtgctgcaaggcgattaagttgggtaacgccagggttttcccagtcacgacgttgtaaaacgacggccagtgaattccatggtctcaactttc

SEQ ID NO: 16 - protein, 676 aa, Dengue virus
MSVTMLLMLLPTALAFHLTTRGGEPHMIVSKQERGKSLLFKTSAGVNMCTLIAMDLGELCEDTMTYKCPRITETEPDDVDCWCNATETWVTYGTCSQTGEHRRDKRSVALAPHVGLGLETRTETWMSSEGAWKQIQKVETWALRHPGFTVIALFLAHAIGTSITQKGIIFILLMLVTPSMAMRCVGIGNRDFVEGLSGATWVDVVLEHGSCVTTMAKDKPTLDIELLKTEVTNPAVLRKLCIEAKISNTTTDSRCPTQGEATLVEEQDTNFVCRRTFVDRGWGNGCGLAGKGSLITCAKFKCVTKLEGKIVQYENLKYSVIVTVHTGDQHQVGNETTEHGTTATITPQAPTSEIQLTDYGALTLDCSPRTGLDFNEMVLLTMEKKSWLVHKQWFLDLPLPWTSGASTSQETWNRQDLLVTFKTAHAMKQEVVVLGSQEGAMHTALTGATEIQTSGTTTIFAGHLKCRLKMDKLTLKGMSYVMCTGSFKLEKEVAETQHGTVLVQVKYEGTDAPCKIPFSSQDEKGVTQNGRLITANPIVTDKEKPVNIEAEPPFGESYIVVGAGEKALKLSWFKKGSSIGKMFEATARGARRMAILGDTAWDFGSIGGVFTSVGKLIHQIFGTAYGVLFSGVSWTMKIGIGILLTWLGLNSRSTSLSMTCIAVGMVTLYLGVMVQA

SEQ ID NO: 17 - protein, 14 aa, Dengue virus
  SIGNAL (1)..(14)
SVTMLLMLLPTALA

SEQ ID NO: 18 - protein, 91 aa, Dengue virus
  misc_feature (1)..(91): pr sequence
  misc_feature (1)..(91): DENV1 pr sequence
FHLTTRGGEPHMIVSKQERGKSLLFKTSAGVNMCTLIAMDLGELCEDTMTYKCPRITETEPDDVDCWCNATETWVTYGTCSQTGEHRRDKR

SEQ ID NO: 19 - protein, 75 aa, Dengue virus
  MISC_FEATURE (1)..(75): M sequence
  MISC_FEATURE (1)..(75): DENV1 M sequence
SVALAPHVGLGLETRTETWMSSEGAWKQIQKVETWALRHPGFTVIALFLAHAIGTSITQKGIIFILLMLVTPSMA

SEQ ID NO: 20 - protein, 495 aa, Dengue virus
  MISC_FEATURE (1)..(495): DENV1 Envelope sequence
MRCVGIGNRDFVEGLSGATWVDVVLEHGSCVTTMAKDKPTLDIELLKTEVTNPAVLRKLCIEAKISNTTTDSRCPTQGEATLVEEQDTNFVCRRTFVDRGWGNGCGLFGKGSLITCAKFKCVTKLEGKIVQYENLKYSVIVTVHTGDQHQVGNETTEHGTTATITPQAPTSEIQLTDYGALTLDCSPRTGLDFNEMVLLTMEKKSWLVHKQWFLDLPLPWTSGASTSQETWNRQDLLVTFKTAHAKKQEVVVLGSQEGAMHTALTGATEIQTSGTTTIFAGHLKCRLKMDKLTLKGMSYVMCTGSFKLEKEVAETQHGTVLVQVKYEGTDAPCKIPFSSQDEKGVTQNGRLITANPIVTDKEKPVNIEAEPPFGESYIVVGAGEKALKLSWFKKGSSIGKMFEATARGARRMAILGDTAWDFGSIGGVFTSVGKLIHQIFGTAYGVLFSGVSWTMKIGIGILLTWLGLNSRSTSLSMTCIAVGMVTLYLGVMVQA

SEQ ID NO: 21 - protein, 676 aa, Dengue virus
  INIT_MET (1)..(1)
  SIGNAL (2)..(15)
  MISC_FEATURE (16)..(106)
  MISC_FEATURE (107)..(181): DENV1 M sequence
  MISC_FEATURE (182)..(676): DENV1 Envelope sequence
MSVTMLLMLLPTALAFHLTTRGGEPHMIVSKQERGKSLLFKTSAGVNMCTLIAMDLGELCEDTMTYKCPRITETEPDDVDCWCNATETWVTYGTCSQTGEHRRDKRSVALAPHVGLGLETRTETWMSSEGAWKQIQKVETWALRHPGFTVIALFLAHAIGTSITQKGIIFILLMLVTPSMAMRCVGIGNRDFVEGLSGATWVDVVLEHGSCVTTMAKDKPTLDIELLKTEVTNPAVLRKLCIEAKISNTTTDSRCPTQGEATLVEEQDTNFVCRRTFVDRGWGNGCGLFGKGSLITCAKFKCVTKLEGKIVQYENLKYSVIVTVHTGDQHQVGNETTEHGTTATITPQAPTSEIQLTDYGALTLDCSPRTGLDFNEMVLLTMEKKSWLVHKQWFLDLPLPWTSGASTSQETWNRQDLLVTFKTAHAKKQEVVVLGSQEGAMHTALTGATEIQTSGTTTIFAGHLKCRLKMDKLTLKGMSYVMCTGSFKLEKEVAETQHGTVLVQVKYEGTDAPCKIPFSSQDEKGVTQNGRLITANPIVTDKEKPVNIEAEPPFGESYIVVGAGEKALKLSWFKKGSSIGKMFEATARGARRMAILGDTAWDFGSIGGVFTSVGKLIHQIFGTAYGVLFSGVSWTMKIGIGILLTWLGLNSRSTSLSMTCIAVGMVTLYLGVMVQA

SEQ ID NO: 22 - protein, 676 aa, Dengue virus; identical to SEQ ID NO: 10
  MISC_FEATURE: DEN2 prM E (F108A)_3' DEN1
  MISC_FEATURE (182)..(477): DEN2 prM E (F108A)
  MISC_FEATURE (182)..(477): DEV2 prM E (F108A)
  MISC_FEATURE (478)..(676): 3' DEV1

SEQ ID NO: 23 - protein, 674 aa, Dengue virus
  misc_feature: DEV3 prM E (F108A)_3'DEV1
  misc_feature (182)..(475): DEV3 prM E (F108A)
  misc_feature (476)..(676): 3' DEV1
MTSLCLMMILPATLAFHLTSRDGEPRMIVGKNERGKSLLFKTASGINMCTLIAMDLGEMCDDTVTYKCPLIAEVEPEDIDCWCNLTSTWVTYGTCNQAGEHRRDKRSVALAPHVGMGLDTRTQTWMSAEGAWRQVEKVETWALRHPGFTILALFLAHYIGTSLTQKVVIFILLMLVTPSMTMRCVGVGNRDFVEGLSGATWVDVVLEHGGCVTTMAKNKPTLDIELQKTEATQLATLRKLCIEGKITNITTDSRCPTQGEAILPEEQDQNYVCKHTYVDRGWGNGCGLAGKGSLVTCAKFQCLEPIEGKVVQHENLKYTVIITVHTGDQHQVGNDTQGVTVEITPQASTVEAILPEYGTLGLECSPRTGLDFNEMILLTMKNKAWMVHRQWFFDLPLPWTSGATTEAPTWNRKELLVTFKNAHAKKQEVVVLGSQEGAMHTALTGATEIQNSGGTSIFAGHLKCRLKMDKLELKGMSYVMCTGSFKLEKEVAETQHGTVLVQVKYEGTDAPCKIPFSSQDEKGVTQNGRLITANPIVTDKEKPVNIEAEPPFGESYIVVGAGEKALKLSWFKKGSSIGKMFEATARGARRMAILGDTAWDFGSIGGVFTSVGKLIHQIFGTAYGVLFSGVSWTMKIGIGILLTWLGLNSRSTSLSMTCIAVGMVTLYLGVMVQA

SEQ ID NO: 24 - protein, 676 aa, Dengue virus
  MISC_FEATURE: DEV4 prM E (F108A)_3'DEV1
  MISC_FEATURE (1)..(477): DEV4 prM E (F108A)
  MISC_FEATURE (478)..(676): 3' DEV1
MSTVTLLCLIPTVMAFHLSTRDGEPLMIVAKHERGRPLLFKTTEGINKCTLIAMDLGEMCEDTVTYKCPLLVNTEPEDIDCWCNLTSTWVMYGTCTQNGERRREKRSVALTPHSGMGLETRAETWMSSEGAWKHAQRVESWILRNPGFALLAGFMAYMIGQTGIQRTVFFVLMMLVAPSYGMRCIGVGNRDFVEGVSGGAWVDLVLEHGGCVTTMAQGKPTLDFELIKTTAKEVALLRTYCIEASISNITTATRCPTQGEPYLKEEQDQQYICRRDVVDRGWGNGCGLAGKGGVVTCAKFSCSGKITGNLVQIENLEYTVVVTVHNGDTHAVGNDTSNHGVTATITPRSPSVEVELPDYGELSLDCEPRSGIDFNEMILMKMEKKTWLVHKQWFLDLPLPWTAGADTSEVHWNHKERMVTFKVPHAKRQDVTVLGSQEGAMHSALTGATEVDSGDGNHMFAGHLKCKVRMEKLRIKGMSYVMCTGSFKLEKEVAETQHGTVLVQVKYEGTDAPCKIPFSSQDEKGVTQNGRLITANPIVTDKEKPVNIEAEPPFGESYIVVGAGEKALKLSWFKKGSSIGKMFEATARGARRMAILGDTAWDFGSIGGVFTSVGKLIHQIFGTAYGVLFSGVSWTMKIGIGILLTWLGLNSRSTSLSMTCIAVGMVTLYLGVMVQA